European Patent Application EP 4 253 955 A1, published October 4, 2023. Title: Extracellular Vesicle (EV) populations in the diagnosis of cancer. Applicant: Albert-Ludwigs-Universität Freiburg. The sequence listing filed with the application follows.

SEQUENCE LISTING (6 sequences)

SEQ ID NO: 1 - DNA, 22 bp, Artificial Sequence
  hAR-FL probe
cgaccatttctgacaacgccaa

SEQ ID NO: 2 - DNA, 23 bp, Artificial Sequence
  hAR-V7 probe
aagcaactgtgtctgtctgaggt

SEQ ID NO: 3 - DNA, 20 bp, Artificial Sequence
  primer
cctccaaggacaattactta

SEQ ID NO: 4 - DNA, 18 bp, Artificial Sequence
  primer
cactgccttacacaactc

SEQ ID NO: 5 - DNA, 18 bp, Artificial Sequence
  primer
caggaagaaactttgctg

SEQ ID NO: 6 - DNA, 22 bp, Artificial Sequence
  primer
catctttatttgtgtattaggc